European Patent Application EP 4 752 233 A1, published June 3, 2026. Title: PREDICTING EFFECTIVENESS OF NEOADJUVANT ANDROGEN DEPRIVATION THERAPY IN PROSTATE CANCER. Applicant: Koninklijke Philips N.V. The sequence listing filed with the application follows.

SEQUENCE LISTING (16 sequences)

SEQ ID NO: 1 - DNA, 9299 bp, Homo sapiens
  source 1..9299: mol_type = genomic DNA
acacttttcctgcgctagagcagcgagcagcctggaacagacccaggcggaggacacctgtgggggagggagcgcctggaggagcttagagaccccagccgggcgtgatctcaccatgtgcggatttgcgaggcgcgccctggagctgctagagatccggaagcacagccccgaggtgtgcgaagccaccaagactgcggctcttggagaaagcgtgagcagggggccaccgcggtctccgcgcctgtctgcaccctgtcgcctgagctgcctgacagtgacaatgacatcccagttaccagtgtccttgaattgatagtggcttctgtttgtcagtctcatataagaactacagctcatcaggaggagatcgcagcagggtaagagacaccaacaccatgttctgcacgaagctcaaggatctcaagatcacaggagagtgtcctttctccttactggcaccaggtcaagttcctaacgagtcttcagaggaggcagcaggaagctcagagagctgcaaagcaaccgtgcccatctgtcaagacattcctgagaagaacatacaagaaagtcttcctcaaagaaaaaccagtcggagccgagtctatcttcacactttggcagagagtatttgcaaactgattttcccagagtttgaacggctgaatgttgcacttcagagaacattggcaaagcacaaaataaaagaaagcaggaaatctttggaaagagaagactttgaaaaaacaattgcagagcaagcagttgcagcaggagttccagtggaggttatcaaagaatctcttggtgaagaggtttttaaaatatgttacgaggaagatgaaaacatccttggggtggttggaggcacccttaaagattttttaaacagcttcagtacccttctgaaacagagcagccattgccaagaagcaggaaaaaggggcaggcttgaggacgcctccattctatgcctggataaggaggatgattttctacatgtttactacttcttccctaagagaaccacctccctgattcttcccggcatcataaaggcagctgctcacgtattatatgaaacggaagtggaagtgtcgttaatgcctccctgcttccataatgattgcagcgagtttgtgaatcagccctacttgttgtactccgttcacatgaaaagcaccaagccatccctgtcccccagcaaaccccagtcctcgctggtgattcccacatcgctattctgcaagacatttccattccatttcatgtttgacaaagatatgacaattctgcaatttggcaatggcatcagaaggctgatgaacaggagagactttcaaggaaagcctaattttgaagaatactttgaaattctgactccaaaaatcaaccagacgtttagcgggatcatgactatgttgaatatgcagtttgttgtacgagtgaggagatgggacaactctgtgaaaaaatcttcaagggttatggacctcaaaggccaaatgatctacattgttgaatccagtgcaatcttgtttttggggtcaccctgtgtggacagattagaagattttacaggacgagggctctacctctcagacatcccaattcacaatgcactgagggatgtggtcttaataggggaacaagcccgagctcaagatggcctgaagaagaggctggggaagctgaaggctacccttgagcaagcccaccaagccctggaggaggagaagaaaaagacagtagaccttctgtgctccatatttccctgtgaggttgctcagcagctgtggcaagggcaagttgtgcaagccaagaagttcagtaatgtcaccatgctcttctcagacatcgttgggttcactgccatctgctcccagtgctcaccgctgcaggtcatcaccatgctcaatgcactgtacactcgcttcgaccagcagtgtggagagctggatgtctacaaggtggagaccattggcgatgcctattgtgtagctgggggattacacaaagagagtgatactcatgctgttcagatagcgctgatggccctgaagatgatggagctctctgatgaagttatgtctccccatggagaacctatcaagatgcgaattggactgcactctggatcagtttttgctggcgtcgttggagttaaaatgccccgttactgtctttttggaaacaatgtcactctggctaacaaatttgagtcctgcagtgtaccacgaaaaatcaatgtcagcccaacaacttacagattactcaaagactgtcctggtttcgtgtttacccctcgatcaagggaggaacttccaccaaacttccctagtgaaatccccggaatctgccattttctggatgcttaccaacaaggaacaaactcaaaaccatgcttccaaaagaaagatgtggaagatggcaatgccaattttttaggcaaagcatcaggaatagattagcaacctatatacctatttataagtctttggggtttgactcattgaagatgtgtagagcctctgaaagcactttagggattgtagatggctaacaagcagtattaaaatttcaggagccaagtcacaatctttctcctgtttaacatgacaaaatgtatgtactcacttcagtacttcagctcttcaagaaaaaaaaaaaaaaccttaaaaagctacttttgtgggagtatttctattatataaccagcacttactacctgtactcaaaattcagcaccttgtacatatatcagataattgtagtcaattgtacaaactgatggagtcacctgcaatctcatatcctggtggaatgccatggttattaaagtgtgtttgtgatagtgtcgtcaaaaaaaaggtttttgaatagaaattacattctttgacaccctcagttctttcaaactttcaactctgcattttattgcattttctcatttaactgttagtatatgtttgaatataggctgactttttttctctattgcactttcttctttttttctttttagaaaataagcaattaggggttagatgcaatatgaatataaaatagttctgtaaataccaaatattatttttagttctggaagttaaaaatactctccatagtaacgtgtgttataataataaatatttcttttgtttgacttttttaaaattctacaatggtaaaagctattttaatccatgttagcaatttaattcctattaattcattttactatcataatagcaaagtattcagaataaaagaggtttatatcttctattaaaatgcagtaatactattcaaatctaatttagctggaagcaacatgggagtaaagtaatcatccaggggacccaccataaaggacattggtaaaacatttacacacgtaaacacacgtgcaggcacacttggaacaatatggacccacttcagcagacatcttctattgccatgctgagctgtttaaagttttaagaagaaaatctaagtatggaagtagaaaataagacttgttcttttggtggatatctcatttttcttgagtatttgtgctgaacattttggtgtatgtctatgaactaagaatcaagtttttgtctcattaaatatacatatatgaagtgtttttattctacttgaaatatcttgacttaaaaaaaacgactgttagtattgatgaagcaaatgaggcagtgactacattatggaaatgtctaagtattttttccggaacttcaactttttctttttgttttacataaacatttaagcagctaggaacttttagttttagttaggtcagttgaagttctctggtgaactaaaaaatctacattttggttggggataaagatttgattttaaaaacagcttgaatttaaagcaagaaaaagatgaacgttatagttttaaaatcaatattagcagagccatagataggctgagctcttatttggggttctgagaaataactcagtttaaaacttctttaactgcctcccttagtacccaggctagcccatggtgacatcagggatattcattactgattggcctctagtattccaagggtactactatagatattacaatgatgctgtttactaagtgataaccccgtatcttacaggactgactttgactcaataaaccactcagcctattattggaaagtgccataggccttgagaaagtatagttacatcctcacaaatatatgaagttaagtcactacttacaaggaaaaaaaatgtaaatacatttttctttctggaaccgaactcttattatggggaaataatagaaataaagaaaatgtaaaagcatgaaatggaatgtagtcttgatcaaacatttcagcagacctcaatttgcttacaatctgtactcaaaaagtttataattcaatcagaattcaaaaagtattttgtgtgtttgtgatgtattagcatatacacaaaacaaatgaggggaatgtatataatcttggtgaaaagttgtatgggagttttttgtacgattcctgcaacttttctataaacgtggcattatatctaaataaaaaattaccaaaaaacatattttcacagtgaagttaaatcatctgtgataggttccccagaccagcctacaaaggcccattaaatacagaataatttgtggatcttcaaagaggatgaacatacatttccatgacagagtccatacgaaattcacaatttagatgctaaaaaatttaaggaatatctttttttctctatcttatctgctttgaagcatagcgattagcgagaaacttttcagatccagaccactgatggtagccagagtagagaccctggagcatagattcttaaaataaataaggggcccaagtcagagctttgaggtattgaagatggaaaaatagtggacaaacagcctgtaatcaggttggggattacgggtactgagttatgttgccatttaactattctaaaaaataagactgggtctcaagactgcttccctaacagactgtttctcctgaaaatgcaggagctattctttctgttctggttatatagtttccattcatggcttcttgtcctgttgttttttgtgtcgagtacactatataaattatctccttatacatatttctcaggcaagcacagagttatactgaacttttctaaagatgctttgcatcaagaagcaaagggaaatacagaattaaaatgtttctttccattttgctttgtttttctatatcgatctagactttgtaggaaaatgcaaagcgtatatttaagaaaacctaaataagaatagattcatttactcattttcatttattcattcatgaagaatttattgaatgcctactatgtgccaggaatattgctatatttttgaaatttaaggataaaatatggcccaatctatcaagaaaggaaagtgaaagacaaatgtaagacataattacaacattctgtgggagcacaaagtaggggactcagttcttagagaagtcttttggtcttagagttcatcaagcagagaaggggaaggacatggtccaggaaaataaatcagcacacaaagagatggggtcttgagggtgcatagtacattctggacagccagttacctgggatgagttgggagggaggagaataaggacaaaagaccatctgggcaaaaatcacgaaggggtatgtgtgtcatgtaaaggtgtgccatgatagttattcatattgctattgtaatattaatatatagtaattaactacacatgacacagctttacatgaccttaagtagttatcaacattaccataatagtaatattaataactacaataagagccattattattcacttgaggcacttgttcaaaatagattttacaaaagaaaaaaaaaaaagaagcaacatgagtaaaattagatccattggctactgactccctctccaacagttttaaagctactagataagagaagcatcaagtcttaaaggaagagaatggtatgatcagatgtgtgttttccaaagactattagaaacagcatggttaaggatagggtggatatttacttgcacaggtgactgaatgaacatctgtttatacatcaagggaaaatgattcattttatatcctggatattttaccataagtatgagcataaagctgggatgtctggcattggaattttatgtcactctcaaggctaattagtctttcagatcctttggtagggaggaaagaagagttgcttcagcattttgactaacatttcttccaaatttcttctccctgatatttccagccacgccaaggcaaagacttcccagctctgtctcaggttaggttaaaagaaggcataggatggaagagggtggtctgtggtaggcctagcaaatgaaagagatgaataaacaagagtgtctagtctaactagtgcctgaggaatagacatcagtcctctgagattacccagctggaaaactgcccagatggagctttacatgcaaagctccagtgaagtctagtgctgtataatgctttaaatccacaatcaagcccttgttgatgcaaatgttagtcgcccaaagcagaatgggttaacgaattactgcagtggttttaggtgcatgggtttgacccatgtaaatcattttaataagtaaaattgaatctttgatacatatttgttgaggagcttgtcagatcactacctttcactgaacagtaaaacatggatcatttatttcacctcattttgcacttcaatgcaatttcactctttaggtggttgtacttggacagttaaatgaagactgtctttaagggtgcagggatggagaacacagcatatatgagaggtgggagggcagagacgccttgcgattcctgtgaggagggacttaccgtctcctccaaaacagaaattcagtgctgcagagacggtagcaaagtgcagttctcttgttaaaacacaggctaaaagcagtgactgcttaacttattaagcagagaaaaccaaaatgtcattttcaaccaaaattgagtgttagagtttatggtctctgttatgatacttttcaagacctgggaaatatttgtatcctttagtgaaaaggggaagaatcaattactgaaagccataagcttacagtaacggagccaattaatcctttgtcatctttgttgagtttagttttcttctgttcttagcacgtcagctagtagatctttgatgaactgttgctcctctttaaatgtttcttttattatattgatgatgtgcactcattcagtattcttattttaagctgcagtaatcactgtacatttgattgccatctgtacttcccttgaagcagctttgcttattacagccacacctgcatctgttttgactagcccacataacctacacatttttcatccaaagctatcccattaccttatttatgtccatttattttcatatatagtatctgccaaaatagtagcaaaagttttatcaatgtgtagatttcaatcagaaaaacctaagcaaaaggaaaaaaaagtgatattctaaaagccacacttcttttatcaccagtgcagttttttccatcatcataaacttagttttatgaaaatgttaatatcttggatttaaacattggggtagaaatcaggacaaaatttaaatgtcatatccaggacttaatctcagatattctggtagaagatatttagataaggttgtggctgcctgtcaagttttttaattttttaaattatataatgtcagaaaattaaatcacaaatgagccttccagattgtgaggaaaattacttggctgaaaatgactttgcataatgcccaaatcttgaagtatctgctcagatgtttgttccatctgaaatgctgccaaatccatctgtattgaggaaagagctatgaggtagtttcagagaaagtgaaaacaaaacaaagcaaaacaaaaatgctattacagaagttggacagcccaatgtgttaagtattatacacctggaacaagagcagcaaaactgaagctctttggaaagttatggcaacagtggtctgggaattctgggcctttagaaataatcattcccagtgatacagggatgtgcagcatccagacactgcttaatcacagtgagctgccgtcttccctgaataagttgtatcttataacattgaagtgaatgaaaatgtattagtatttgagaatttactattccttcacctccttgcacatgtaaattaaagatgttttggaaaatatgagaacttgatgttcactgccctagagcactattctccaaccttttagattcctgcaatctgttaataaaatattgtaggacaacaactctatagactgatacatgctgctctcaatccatatactacatattaggacagcttttcttttctaaatgagcatgaatataaatagaaattctagtattttcttcacctaccccagtgaatcatctttatattttacttgggaaactgctacagttggctagtgggtcttcacttttattgctttgagaaatggataaaagacatagactatcacccctccaaaaatgtgcatatggccccatacaagacacatgtactgccagagcttggggaactccctagaatctactcctagaccaccctagtgaagtaccatagaccatattgtctagatgggacaaaataataaattttgactaagaacttactgtttagagagaaaaaatagtaaataatgttcaaaatgagaagacaataactgacaagtctgtgatttttgggttagatgagaccacttttgatttttgaggaataaaaggagttagttttttggtcctgatgtgtaaaatgattcatggggtttcacatacagacaagtagttttcttttcagcaaatatttaacatatctctcaatatatttttcaccagtttttggtaaatatgcattgctataggtataccaagttttttttgttatgtttagtaactaatttcattttttctgtatatgtaaatatagctattggaccctgcattgaaaaccttcttagtactaacaacactccttttattattaccttcatagttactttaaatgacatatttatttcgagttttacttctggctgagttgcaaagtctatgagaatgttacctcctgtctcagaagcttgttagttattgtgccacctaaatattgtaataaaagtgtttaaataaaaatcttcttaaaatttaaaa

SEQ ID NO: 2 - protein, 690 aa, Homo sapiens
MFCTKLKDLKITGECPFSLLAPGQVPNESSEEAAGSSESCKATVPICQDIPEKNIQESLPQRKTSRSRVYLHTLAESICKLIFPEFERLNVALQRTLAKHKIKESRKSLEREDFEKTIAEQAVAAGVPVEVIKESLGEEVFKICYEEDENILGVVGGTLKDFLNSFSTLLKQSSHCQEAGKRGRLEDASILCLDKEDDFLHVYYFFPKRTTSLILPGIIKAAAHVLYETEVEVSLMPPCFHNDCSEFVNQPYLLYSVHMKSTKPSLSPSKPQSSLVIPTSLFCKTFPFHFMFDKDMTILQFGNGIRRLMNRRDFQGKPNFEEYFEILTPKINQTFSGIMTMLNMQFVVRVRRWDNSVKKSSRVMDLKGQMIYIVESSAILFLGSPCVDRLEDFTGRGLYLSDIPIHNALRDVVLIGEQARAQDGLKKRLGKLKATLEQAHQALEEEKKKTVDLLCSIFPCEVAQQLWQGQVVQAKKFSNVTMLFSDIVGFTAICSQCSPLQVITMLNALYTRFDQQCGELDVYKVETIGDAYCVAGGLHKESDTHAVQIALMALKMMELSDEVMSPHGEPIKMRIGLHSGSVFAGVVGVKMPRYCLFGNNVTLANKFESCSVPRKINVSPTTYRLLKDCPGFVFTPRSREELPPNFPSEIPGICHFLDAYQQGTNSKPCFQKKDVEDGNANFLGKASGID

SEQ ID NO: 3 - DNA, 3283 bp, Homo sapiens
  source 1..3283: mol_type = genomic DNA
ccagattgctcttctgggcgtgggagaaggttctgtctatcagtgctgcgagaaaggaaagaaacaagtttgctctcagcggatctttaaatggatgagatggctaccactcagatttccaaagatgagcttgatgaactcaaagaggcctttgcaaaagttgatctcaacagcaacggattcatttgtgactatgaacttcatgagctcttcaaggaagctaatatgccattaccaggatataaagtgagagaaattattcagaaactcatgctggatggtgacaggaataaagatgggaaaataagttttgacgaatttgtttatatttttcaagaggtaaaaagtagtgatattgccaagaccttccgcaaagcaatcaacaggaaagaaggtatttgtgctctgggtggaacttcagagttgtccagcgaaggaacacagcattcttactcagaggaagaaaaatatgcttttgttaactggataaacaaagctttggaaaatgatcctgattgtagacatgttataccaatgaaccctaacaccgatgacctgttcaaagctgttggtgatggaattgtgctttgtaaaatgattaacctttcagttcctgataccattgatgaaagagcaatcaacaagaagaaacttacacccttcatcattcaggaaaacttgaacttggcactgaactctgcttctgccattgggtgtcatgttgtgaacattggtgcagaagatttgagggctgggaaacctcatctggttttgggactgctttggcagatcattaagatcggtttgttcgctgacattgaattaagcaggaatgaagccttggctgctttactccgagatggtgagactttggaggaacttatgaaattgtctccagaagagcttctgcttagatgggcaaactttcatttggaaaactcgggctggcaaaaaattaacaactttagtgctgacatcaaggattccaaagcctatttccatcttctcaatcaaatcgcaccaaaaggacaaaaggaaggtgaaccacggatagatattaacatgtcaggtttcaatgaaacagatgatttgaagagagctgagagtatgcttcaacaagcagataaattaggttgcagacagtttgttacccctgctgatgttgtcagtggaaaccccaaactcaacttagctttcgtggctaacctgtttaataaatacccagcactaactaagccagagaaccaggatattgactggactctattagaaggagaaactcgtgaagaaagaaccttccgtaactggatgaactctcttggtgtcaatcctcacgtaaaccatctctatgctgacctgcaagatgccctggtaatcttacagttatatgaacgaattaaagttcctgttgactggagtaaggttaataaacctccatacccgaaactgggagccaacatgaaaaagctagaaaactgcaactatgctgttgaattagggaagcatcctgctaaattctccctggttggcattggagggcaagacctgaatgatgggaaccaaaccctgactttagctttagtctggcagctgatgagaagatataccctcaatgtcctggaagatcttggagatggtcagaaagccaatgacgacatcattgtgaactgggtgaacagaacgttgagtgaagctggaaaatcaacttccattcagagttttaaggacaagacgatcagctccagtttggcagttgtggatttaattgatgccatccagccaggctgtataaactatgaccttgtgaagagtggcaatctaacagaagatgacaagcacaataatgccaagtatgcagtgtcaatggctagaagaatcggagccagagtgtatgctctccctgaagaccttgtggaagtaaagcccaagatggtcatgactgtgtttgcatgtttgatgggcaggggaatgaagagagtgtaaaataaccaatctgaataaaacagccatgctcccaggtgcatgattcgcaggtcagctatttccaggtgaagtgcttatggcttaaggaactcttggccattcaaaggacttttcattttgattaacaggactagcttatcatgagagccctcaggggaaagggtttaagaaaaacaactcctctttcccatagtcagagttgaatttgtcaggcacgcctgaaatgtgctcatagccaaaacattttactctctcctcctagaatgctgcccttgacatttcccattgctgtatgttatttcttgctctgttatcttttgccctcttagaatgtccctctcttgggacttgcttagatgatgggatatgaatattattagacagtaattttgctttccatccagtatgctagttcttattcgagaactatggtcagagcgtatttggatatgagtatcctttgcttatctttgtagtactgaaaatttgccgaagtaactggctgtgcagaatgtaatagaagcttttcttattcttttattcttaagatcagtatctttttacagtattctttctacatgatccttttttgtacatttaagaatattttgattatattaaacaagactgctgattttgctactttttttaaggggtcttcaagtaagtaaaacatacatcgtagctagaagaaaaatgtaccttaaatttgcatcttccctctcatacccaagctgtaaacaattgaaatattttgtcttaaatcacttggttcaatacatgcttatttgttttaaaacctgtatcatcaaactctctctctaaatttaaaatgctgttgaatatgatacttttgaggagagagtgtgctcagaacttagacgggatttggtaggccaagtatgctaagtgtacaatatattttttaattttacacctgaaacaaagaaatgtggtcactaaaaataaaagtatatatgtaggaattaatgtactcttgctttgtcaagctgtttgctatagtttccaaggtattatgttactctaactctgaaaagtgatgtaatctggtagcaatgtagtagttcaaataaaggcatttacataataattagtctgttcttcatgcttttgtctcttaggaagtatgccaatgtttgtcaggatttttttctttttgtttttctgatgtattctgtaaaatggtgtttgttaaatttgagttttgggagctgaattagaggtactgaattaaggacagtacaaatgaagtaaaaaggttttctccaatttaccaaaa

SEQ ID NO: 4 - protein, 630 aa, Homo sapiens
MDEMATTQISKDELDELKEAFAKVDLNSNGFICDYELHELFKEANMPLPGYKVREIIQKLMLDGDRNKDGKISFDEFVYIFQEVKSSDIAKTFRKAINRKEGICALGGTSELSSEGTQHSYSEEEKYAFVNWINKALENDPDCRHVIPMNPNTDDLFKAVGDGIVLCKMINLSVPDTIDERAINKKKLTPFIIQENLNLALNSASAIGCHVVNIGAEDLRAGKPHLVLGLLWQIIKIGLFADIELSRNEALAALLRDGETLEELMKLSPEELLLRWANFHLENSGWQKINNFSADIKDSKAYFHLLNQIAPKGQKEGEPRIDINMSGFNETDDLKRAESMLQQADKLGCRQFVTPADVVSGNPKLNLAFVANLFNKYPALTKPENQDIDWTLLEGETREERTFRNWMNSLGVNPHVNHLYADLQDALVILQLYERIKVPVDWSKVNKPPYPKLGANMKKLENCNYAVELGKHPAKFSLVGIGGQDLNDGNQTLTLALVWQLMRRYTLNVLEDLGDGQKANDDIIVNWVNRTLSEAGKSTSIQSFKDKTISSSLAVVDLIDAIQPGCINYDLVKSGNLTEDDKHNNAKYAVSMARRIGARVYALPEDLVEVKPKMVMTVFACLMGRGMKRV

SEQ ID NO: 5 - DNA, 5145 bp, Homo sapiens
  source 1..5145: mol_type = genomic DNA
actagcggcgcccgggcgcggagtgcgcagggcaaggtcctgcgctctgggccagcgctcggccatgcgatccgccgcgcggaggggacgcgccgcgcccgccgccagggactctttgccggtgctactgtttttatgcttgcttctgaagacgtgtgaacctaaaactgcaaatgcctttaaaccaaatatcctactgatcatggcggatgatctaggcactggggatctcggttgctacgggaacaatacactgagaacgccgaatattgaccagcttgcagaggaaggtgtgaggctcactcagcacctggcggccgccccgctctgcaccccaagccgagctgcattcctcacagggagacattccttcagatcaggcatggacgccagcaatggataccgggcccttcagtggaacgcaggctcaggtggactccctgagaacgaaaccacttttgcaagaatcttgcagcagcatggctatgcaaccggcctcataggaaaatggcaccagggtgtgaattgtgcatcccgcggggatcactgccaccaccccctgaaccacggatttgactatttctacggcatgcccttcacgctcacaaacgactgtgacccaggcaggccccccgaagtggacgccgccctgagggcgcagctctggggttacacccagttcctggcgctggggattctcaccctggctgccggccagacctgcggtttcttctctgtctccgcgagagcagtcaccggcatggccggcgtgggctgcctgtttttcatctcttggtactcctccttcgggtttgtgcgacgctggaactgtatcctgatgagaaaccatgacgtcacggagcaacccatggttctggagaaaacagcgagtcttatgctaaaggaagctgtttcctatattgaaagacacaagcatgggccatttctcctcttcctttctttgctgcatgtgcacattccccttgtgaccacgagtgcattcctggggaaaagtcagcatggcttatatggtgataatgtggaggagatggactggctcataggtaaggttcttaatgccatcgaagacaatggtttaaagaactcaacattcacgtatttcacctctgaccatggaggacatttagaggcaagagatggacacagccagttagggggatggaacggaatttacaaaggtgggaagggcatgggaggatgggaaggtgggatccgcgtgcccgggatcttccactggccgggggtgctcccggccggccgagtgattggagagcccacgagcctgatggacgtgttccctactgtggtccagctggtgggtggcgaggtgccccaggacagggtgattgatggccacagcctggtacccttgctgcagggagctgaggcacgctcggcacatgagttcctgtttcattactgtgggcagcatcttcacgcagcacgctggcaccagaaggacagtggaagcgtctggaaggttcattacacgaccccgcagttccaccccgagggagcgggggcctgctacggccgaggcgtctgcccatgctccggggagggcgtgacccatcacagaccccctttgctctttgacctctccagggacccctccgaggcacggcccctgacccccgactccgagcccctgtaccacgccgtgatagcaagggtaggtgccgcggtgtcggagcatcggcagaccctgagtcctgtgccccagcagttttccatgagcaacatcctgtggaagccgtggctgcagccgtgctgcggacatttcccgttctgttcatgccacgaggatggggatggcaccccctgaatgccaggactgtgagagaggatccaggagagcctgactgcgttgcaaacaaaattctccaagcttggttctatcttcagcttccctttttgcaaggaacatgccctggactgagagtgggtccccactttctttctttctttctttcttttttgagacagagtgtcgctctgtccctcaggctggaatgcaatggcacgatctctgctcactgcaacctccgcctcccgggttcaagcgattttcctgcctcagcctcctgagtacccaggattacaggcaccaggcacctgccaccatgcctagctaatttttgtagttttagtagagacagggtttcaccatgttgcccaggctggtctcgcactcctgacctcaagtcatccacctgcctcagcctcccaaagtgctgggattacaggcacgagccactgcgcccatgtagggtttccctttcctgatttgtgaaataagactgtcccagtaggcacccactgatgcctcctcttcctcttctaaatctcagggttcgtcattgtgccaatgcccgatgttttcacccctccgtcttaaagcattgttgcaatttcatcacctagatgacataacagccttacaaaaggacagggaggagtgtctgttcctactctcacatagcggaggaaagttagagcctctcagtctctgtttatgaggactcattaatctcaaataattgatgcatttttcatacattagggtctctgtccatgtgtcttcctgatattgttatagaaatggcttcaggctgctggtaacagatgctgcggaaaaagaatgccttaaacaaagccaggcacggtgactcacacctgtaatcccagcactttgggaggctaaggtgggaggatcacttgagcctaggagttagacacctacccagcctgagcaacacagtgagacctcatctctacaaaaaacaaataattagctagatgtcgtggcgcacagctgtagtctcagctacttaggaggctgaggcgggaggattatttgagcctgggaggtcaaaactgcaatgagctaagattgcactactgcactccgggctgggagacagagtaagaccctgccttaaaaaaaaaaaaaaaaaaatgccttaaagaaaataataagagaagggtgtgttctcttccaagtaatgagccgatcaaggggaagcaacccaaggctagcaggctcttttcaattcccagctctgccactcttagcatggcagagagttggcctcattatgccagtatggctgccacagtgtcagacatcacattccaggcagtggaaaggagaaagaaccaaagggcatccctttctcttgaagcagtccctgtgaggggggattatctggaagccccaacccaatttctgcttccaaccattatccatagaaacaactggaagttgagaagtgcagtcttttaggtgggcacctggctgccctgtatgaaaccagaattaggttggtcagcaggaaaacaagaaaacacttactgtgttgactgaggtttttgacgcatcgctttattgtcaaattaaacaactctatctcattctgcactgaaacacgtactaccattgcctataattggaaaatgatcctcagaggcacagaagatgccctgatggaaagtttgccccttgggcaaagagacagccatgggaaccttcagacatagagagagaaggtggcttttctccctacattcctcaaatagctaagatttggccagtgtgttttctaagtcaattctagtgtgtttcatcctcacctcttccctctgtggctttgatgatggaagtgtagtcctaacctactgcacagctgggaccccctgcccctagatcccaatactggggatgggaggaccttgcactattcccctcagtccatctatcgaggtctttgcaggaagcatactgggaattgaaacgagagcctaaatgacatctaagaaaggcagtgttcaataccaggtattaggtgaggatgggattctaaggacatcagtgggaggcagggagccaccttcagacctcagcatggaagcttccaagatccagaggaagaggcaacagcactgagagtcataggtagaagaatcatcacagccctgctaaccaggcagctgatgcccctctcccctggctccctgtgtccaaatcctacaggggcatctgttggctgaactcaacctgaagccaaagagaagatgagtggagagaggcaacatttatagagctcaggtttctagggctggagagggatctggagggacacacaggagacacctggcataaccaaaaaatgattaaaaaaaaaaaaaaaaagaaacatctatggagcatgggacacggggagtggaggcagctaaaagccatctcatctttcaccgtattcaacaagcccattataacaagtctttcacgctcaaccattcaaacaatcccaacaatcccagcctaagaatttcctggcatttgatgaaaatggctgtgggttttgctatctttaagctccctgggaagcaggatataagcccagggctggcaggctctttctagctacctgctcttgcacatagagtttgcctcatggttgcaagaaggctgccatagctccagatggcacatagacattccaggcagcaggaaaaaggaaggagcacttaaccgaaggaggtcagggagttggttagtctccacctgaagaagagagccatgaaccagcttcagttgactaacgggctcctgtgagtgcatctttggacttttctggaggttgaaatctagatgtggtatgtgtcttaaagcagccaccaactcctcccattaccttccaagtgagcccaactacacgatggagcctcttccctgcccttggatctgggctgagcctctgacttgcgttgaccaacagaatgcagtgaaagtgatgccgatactaccctccctgccctagacttgggatacctggcagctatattcttccattcctcaggacttgcaaaaacgggtctcagcatgccttcccagagccatgaggtgtttctttgcccattcattgatctgagaagtgagtgtaaggagtttaaatcaacctctgttctgtgctagttaaggtaataaagttgctgcagtccagggggtaggtacctgtggacggctctgcgaataggacagttgcatttcttgggaatcaagtgcatccctaggctggcagtgcagcagaaatactgaataaaatgtgacaaatctccctg

SEQ ID NO: 6 - protein, 593 aa, Homo sapiens
MRSAARRGRAAPAARDSLPVLLFLCLLLKTCEPKTANAFKPNILLIMADDLGTGDLGCYGNNTLRTPNIDQLAEEGVRLTQHLAAAPLCTPSRAAFLTGRHSFRSGMDASNGYRALQWNAGSGGLPENETTFARILQQHGYATGLIGKWHQGVNCASRGDHCHHPLNHGFDYFYGMPFTLTNDCDPGRPPEVDAALRAQLWGYTQFLALGILTLAAGQTCGFFSVSARAVTGMAGVGCLFFISWYSSFGFVRRWNCILMRNHDVTEQPMVLEKTASLMLKEAVSYIERHKHGPFLLFLSLLHVHIPLVTTSAFLGKSQHGLYGDNVEEMDWLIGKVLNAIEDNGLKNSTFTYFTSDHGGHLEARDGHSQLGGWNGIYKGGKGMGGWEGGIRVPGIFHWPGVLPAGRVIGEPTSLMDVFPTVVQLVGGEVPQDRVIDGHSLVPLLQGAEARSAHEFLFHYCGQHLHAARWHQKDSGSVWKVHYTTPQFHPEGAGACYGRGVCPCSGEGVTHHRPPLLFDLSRDPSEARPLTPDSEPLYHAVIARVGAAVSEHRQTLSPVPQQFSMSNILWKPWLQPCCGHFPFCSCHEDGDGTP

SEQ ID NO: 7 - DNA, 6741 bp, Homo sapiens
  source 1..6741: mol_type = genomic DNA
acattcgctttttatttgccggtggtgctgctgacgggccctcggagcggggctgtgtctggacacttctgggagccttggacggctctggagaggaggcaggagctgcccaggaaggagcttaattccgtcgcttctgagctgtctgcacggcaggaggagagtgaacattctcataaacatttaattgaactccgccgggaatttaagaaaaatgtacctgaggaaatcagagagatggtggctcctgtattaaaaagcttccaagccgaggtggtggcccttagtaagagaagtcaggaggcggaggctgcttttctgagtgtttacaagcaattaattgaagcaccagaccccgtgcctgtgtttgaggcggcacgcagcctagacgacagactgcagccccccagctttgaccccagtgggcagccccggcgagacctccacacttcgtggaagaggaaccccgagctcctcagccccaaagagcagagagaggggacgtcgcctgccgggcccacgctgaccgagggaagccgcctcccaggcattcccgggaaagccctcctgacagaaaccttgctgcagagaaatgaggcggaaaaacaaaagggccttcaagaagtacagatcactttggcggccagactgggggaggcagaggagaaaatcaaagtcctacattcagcgctaaaggctacgcaggcagagctgctagagctgcggcggaagtacgacgaggaggcagcatccaaggcagatgaagtcggcctgatcatgaccaacctggagaaagctaatcagcgagctgaggctgcccagcgggaggtggaaagtctccgggaacagctggcctctgtcaacagctccatccgcctggcttgctgctctccccaggggcccagtggggataaggtgaacttcactctgtgctcgggccctcggctggaggccgcgctggcctccaaggacagggagatcctgcggctgctgaaggacgtgcagcacctccagagctcactgcaggagctggaggaggcatccgccaaccagatcgccgacctggagcggcagctcacggccaagtccgaggccatagaaaagctggaagagaagctccaggcccagtctgactatgaggaaattaaaacggagctgagcatcctgaaagccatgaagctggcctccagcacctgcagcctcccccagggcatggccaagcctgaagactcactgcttattgcaaaggaggccttcttccccacgcagaaattccttctggagaagcccagcctcctggccagccctgaggaagacccatcagaggacgattccatcaaggattcactgggcacggagcagtcctacccctcccctcagcagctcccacctccaccagggccagaagaccccctgtctcccagccccgggcagcccctgctgggccccagcttggggcctgacggcactcggactttctcgctgtcccccttccccagcctggcatcaggggagagactgatgatgcccccagccgccttcaagggagaggcgggcggcctgctggtgttccccccagccttctatggcgccaagccccccacagcccctgccaccccggcccctggccctgagccactgggcggtcctgagcccgcggatggtggtgggggcggagcggcggggcccggggcagaggaggagcagctggacacggcagagatcgccttccaggtgaaggagcagctgctgaaacacaacatcgggcagcgggtgtttgggcattacgtgctggggctgtcgcagggctcggtcagcgagatcctagcccggcccaagccctggcgcaagctcacggtgaagggcaaggagcccttcatcaagatgaagcagttcctgtcggatgagcagaatgtactggcgctcaggaccatccaagtgcggcagcgaggcagcatcaccccgagaatccgcacgcctgagacaggctcagacgacgccatcaagagcattctagagcaggccaagaaggagatcgagtcgcagaagggcggcgagcccaagacctcggtggccccgctgagcatcgccaacggcacgacccccgccagcacctcggaggacgccatcaagagcatcctggagcaggcacgccgtgagatgcaggcgcaacagcaggcgctgctggagatggaggtggcgcccaggggccgctcggtgcccccctcgcccccggagcggccatcactggccaccgcgagccagaacggggccccggccttggtgaagcaggaggagggcagcgggggccccgcgcaggcgccgctcccggtcctgtcccccgccgccttcgtgcagagcatcatccgcaaggtcaagtccgagatcggcgacgccggctacttcgaccaccactgggcctccgaccgcggcctgctcagccgcccctacgcctccgtgtcgccctcgctgtcctcctcctcctcctctggctactctggccagcccaacggccgcgcctggccccgcggggacgaggcccctgtgccccccgaggacgaggcggcggcaggggcggaggacgaaccccccaggacgggcgagctcaaggctgagggcgcgacggccgaggcgggcgcgcggctgccctactacccggcctacgtgccgcgcaccctgaagcccaccgtgccgccgctgacccccgagcagtacgagctgtacatgtaccgtgaggtagacacgctggagctcacccgccaggtcaaggagaagctggccaagaacggcatctgccagaggatcttcggggagaaggtgctgggcctgtcacagggcagcgtgagcgacatgctgtcccggccgaagccatggagcaagctgacgcagaaggggcgggagcccttcatccgcatgcagctgtggctctctgaccagctcggccaggcagtgggccagcagcctggtgcctcccaggccagtcccacagaaccaaggtcctcaccatccccaccccccagccccacagagcctgagaagagctcccaggagccgttgagcctgtccctggagagcagcaaggagaaccagcagccagagggccgctccagctcctcgttgagcgggaagatgtactcaggcagccaggccccagggggcatccaggagatcgtggccatgtcccccgagctggacacgtactccatcaccaagagggtgaaggaggtcctcacagacaacaatctagggcagcggctgtttggggaaagcatcctgggtctgacacagggctccgtgtctgacctgctgtcccggcccaaaccctggcacaagctgagcctgaaggggcgggagccttttgtccgcatgcagctgtggctcaatgacccccataacgtggagaagctgagggatatgaagaagctggagaagaaagcctacctgaaacgtcgctatggcctcatcagcaccggctcagacagtgagtccccggccacccgctcagagtgccccagcccctgcctgcagccccaggacctgagcctcctgcagatcaagaagccccgggtggtgctggcacccgaggagaaggaggcactgcggaaggcctatcagctggaaccctacccctcgcagcagaccatcgagctcctctccttccagctcaacctcaagaccaacaccgtcatcaactggttccacaactacaggtcccggatgcgccgggagatgttggtggaggggacccaggatgagccagaccttgatccaagcgggggtcctggaatcctaccgccaggccactcccacccagaccccaccccgcagagccctgactctgagactgaggaccagaagccaaccgtgaaggaactggagcttcaggagggccctgaggagaacagcacacccctgaccacccaggacaaggcccaagtgaggatcaagcaggaacagatggaggaggatgctgaggaagaggcaggcagccagccccaggactcaggggagctggacaaaggccaaggtccccccaaagaggagcatcccgaccctccgggtaatgatggactcccaaaagtggctcccgggcccctccttccaggtggatccaccccagactgtccctcacttcatccccaacaggagagtgaggccggggagcgacttcacccggaccctttaagttttaagtcagcctcagagtcctcacgctgcagcctggaggtgtcactgaactcgccctcggccgcctcctcaccaggcctcatgatgtctgtgtcacctgtcccctcctcctcagctcccatctccccatccccacctggcgccccccctgccaaagtgccgagtgccagccccactgctgacatggctggagccttgcaccccagtgccaaggtgaaccccaacttgcagcggcggcatgagaagatggccaatctgaacaacatcatttaccgagtagagcgggctgccaatcgggaggaggccctggagtgggagttctgaaggcagggtgagggggcaagggacataccctggtaactaccttccttctcgcacttactctcctcaacaggatggggtaagggagggaggaactcaaccatcaaaatgtggacagcaatgttatgccgtttacgttttttgttgtaatcctagttctatgaagctgtgtgagcaggtgggtcaaatgccattgcctccacttttctgcacccccctgctcctcttcaccctgacccctctgcaggaggcagaagcaaaatggcaccacatattcacctgaaaactccaaactcttttagaaaaataaataaatatttatagacctcttttagatattttaataaaggatcctttggaatttatcccagctgatgctgttttgatattacagagagttataaaatcaggatgctgtcacaactgttgcgaagtatacactgaagttgtgtcgtttttgccactagatgagattaaaagaagacaattattcaaagccatcacaaaacactataagactgaccaaaatttagataacctttgaaccacgatttttttccacatctgtctgtgagacacagcgcaatgctactgcccttccagaaactgtgctaaaaagagaaagtccaaaagactctaaacaaaaacctcgacgccgttgaggatgtgtttcattctggtggtctgttttgcaagcttgataacagaatgtccgtgccattgtaaatgttgtagagatgtgggccgtggcccaaccgtcctatatgagatgtagcatggtacagaacaaactgcttacacaggtctcactagttagaaacctgtgggccatggaggtcagacatccatcttgtccatctataggcaagaagtgtttccagatcctttggaaaggtgggcatggggcaggtgcttggagagtggcgtttgagccagagcgaccccatttcccgtgtgaaccataggcacaacccaggaagtttccccacttgtaggagtgtgggtattccagagcaagactgtggccaccatcttcccctcttggtgttttccgaaagtgacagtgttggtcatcccatgaccactgaagcttagtaaccagcgccaaaaagtagattcatcaaactagagaccccagctccccttctcgccatcttctttctcaagttgaccgtggtgctgtttctggaaggcatctgcaactccaagtccatgcagaactctggaaggccaagttcatcgcagcatgttcaccatatcccagcctccaaatctatcctcctaccttccaacgcatgacctgttggggagcagagacttaacccccaactcagaggaacccttcctccagcgtctttggcatggtttctagggtgagagttcccaatttggatagaacggccaccatattggttactgaatctctctcccttgtttttattacgtttcctttttcaaactgtccatgggaaggctgaattgagtgactccccagaatgaagatgagaaggtgaatataatcaatgccaatgtaatgccagcgggtgagatggccgatggaggtttcaaagatgtagctagcattttgaaaccatatgggcaaaacccggcaaccagaaggggacagataaggaccgttccagaaatcccaactctcacacccagcccaggctgcagtctccacaccaaacagtcaacaaaacacaaaccctgaaggaaaaccttttccatacacccaggctatgcattgaagagttttccactgtatacatttttatccagatgaaggtatttttatattttgacaataggaaacagtgaccattttcagagtaatcaaatctggaacaaatgaaacatcttttagccaccaccaccctgttgcaattaagacaaccgtgggggaacacaccactttttactgttgaaaccaacacaacgttgaaatccaggcttatacgcagactccgattcctagagaactaaatttggctttagtgtgacgggatttgattaagcacttagtatagtcttttgaacacggaaatcctgttgtacttaaagctagcggacccgtgaacaactttgtcaggttcacgtcctataacggttaaaaaacacacacacacatacacaaaccgtttctatgagagattgatgaactttgtttaaaattttaaaaaaaggaacacgttctgtaaacgagtcgctaaatacagaattgtataataa

SEQ ID NO: 8 - protein, 1424 aa, Homo sapiens
MVAPVLKSFQAEVVALSKRSQEAEAAFLSVYKQLIEAPDPVPVFEAARSLDDRLQPPSFDPSGQPRRDLHTSWKRNPELLSPKEQREGTSPAGPTLTEGSRLPGIPGKALLTETLLQRNEAEKQKGLQEVQITLAARLGEAEEKIKVLHSALKATQAELLELRRKYDEEAASKADEVGLIMTNLEKANQRAEAAQREVESLREQLASVNSSIRLACCSPQGPSGDKVNFTLCSGPRLEAALASKDREILRLLKDVQHLQSSLQELEEASANQIADLERQLTAKSEAIEKLEEKLQAQSDYEEIKTELSILKAMKLASSTCSLPQGMAKPEDSLLIAKEAFFPTQKFLLEKPSLLASPEEDPSEDDSIKDSLGTEQSYPSPQQLPPPPGPEDPLSPSPGQPLLGPSLGPDGTRTFSLSPFPSLASGERLMMPPAAFKGEAGGLLVFPPAFYGAKPPTAPATPAPGPEPLGGPEPADGGGGGAAGPGAEEEQLDTAEIAFQVKEQLLKHNIGQRVFGHYVLGLSQGSVSEILARPKPWRKLTVKGKEPFIKMKQFLSDEQNVLALRTIQVRQRGSITPRIRTPETGSDDAIKSILEQAKKEIESQKGGEPKTSVAPLSIANGTTPASTSEDAIKSILEQARREMQAQQQALLEMEVAPRGRSVPPSPPERPSLATASQNGAPALVKQEEGSGGPAQAPLPVLSPAAFVQSIIRKVKSEIGDAGYFDHHWASDRGLLSRPYASVSPSLSSSSSSGYSGQPNGRAWPRGDEAPVPPEDEAAAGAEDEPPRTGELKAEGATAEAGARLPYYPAYVPRTLKPTVPPLTPEQYELYMYREVDTLELTRQVKEKLAKNGICQRIFGEKVLGLSQGSVSDMLSRPKPWSKLTQKGREPFIRMQLWLSDQLGQAVGQQPGASQASPTEPRSSPSPPPSPTEPEKSSQEPLSLSLESSKENQQPEGRSSSSLSGKMYSGSQAPGGIQEIVAMSPELDTYSITKRVKEVLTDNNLGQRLFGESILGLTQGSVSDLLSRPKPWHKLSLKGREPFVRMQLWLNDPHNVEKLRDMKKLEKKAYLKRRYGLISTGSDSESPATRSECPSPCLQPQDLSLLQIKKPRVVLAPEEKEALRKAYQLEPYPSQQTIELLSFQLNLKTNTVINWFHNYRSRMRREMLVEGTQDEPDLDPSGGPGILPPGHSHPDPTPQSPDSETEDQKPTVKELELQEGPEENSTPLTTQDKAQVRIKQEQMEEDAEEEAGSQPQDSGELDKGQGPPKEEHPDPPGNDGLPKVAPGPLLPGGSTPDCPSLHPQQESEAGERLHPDPLSFKSASESSRCSLEVSLNSPSAASSPGLMMSVSPVPSSSAPISPSPPGAPPAKVPSASPTADMAGALHPSAKVNPNLQRRHEKMANLNNIIYRVERAANREEALEWEF

SEQ ID NO: 9 - DNA, 3968 bp, Homo sapiens
  source 1..3968: mol_type = genomic DNA
ggcggaagcgggagcctctgtcggccgcggaagcctggagtgggcggtacgcagacgcgcgcggtgagacccgctgtctgctcagcggactctgcccgcccccacctccccctgcgtcgggccgacatgaaggactcgctggtgctgctgggccgtgtcccggcgcacccggactcccgctgctggttcctggcctggaaccccgcggggaccctgctggcctcgtgcggcggcgaccggagaatccgcatctggggcacggagggtgacagctggatctgcaagtctgtcctttctgaaggccaccagcgcaccgtgcggaaggtagcctggtccccctgcggtaattacctggcctctgccagctttgatgctaccacttgcatttggaagaagaaccaggatgactttgagtgtgtaaccactctcgagggccatgaaaatgaggtcaagtcagtggcttgggccccatctggcaacctcctggccacttgcagccgagataagagcgtttgggtctgggaagttgatgaagaggatgagtatgaatgtgtcagtgttctcaactcccacacacaggatgtcaagcatgtggtttggcacccaagtcaggagctcttagcttctgccagctatgatgacacagtgaagctgtaccgggaggaagaggatgactgggtatgctgtgccacccttgagggccatgaatccactgtgtggagcttggcctttgacccgagtggccagcgcctggcgtcttgtagtgatgaccgtactgtgcgtatctggcgtcagtatctaccaggcaatgaacaaggggtggcatgcagcggctctgaccccagttggaaatgtatctgtactttgtccggcttccactcaaggaccatttatgacattgcttggtgtcagctgacaggggctctggccacagcttgtggggatgacgcgatccgcgtgtttcaggaggatcccaactcggatccacagcagcccaccttctccctgacagcccacttgcatcaggcccattcccaggatgtcaactgtgtggcctggaaccccaaggagccagggctactggcctcctgcagtgatgatggggaggtggccttctggaagtatcagcggcctgaaggcctctgagctacctcgactttggacagagtaatgactccccagaaaacgtcatataagactttaccagcccctgagaggaccaggaggagcatccttgaccttcatttaacttggctcacttctcttcagacttgggtagaagtgcagagccacagaattgctttccttccccgcctttgacatgaggccttcagtaaagagctacagaacatgagtacattgttataccacagatttttcttgcattagggcacagtgttaaattttttggaggtaaatatactatttataatcactatatatagtaggagggggtatgtgtctcaggcttttctgaagttgcaagacttaaagaaataatccatctgcatcccaagtcctattttataaggatattcataaaaattccatggtgaatccttgtctgaaataggtcctcccttcccagtttctgtgtaagtctttgcatttaagacatccaatcaataatgaaggaaatttttttctgaatgtaggtttgagtgaggggcacctctgctttcccttagcaaccctcatatacctccctgcaccgttacgctgtgatggcaactggggatagaaaaaaaatggggaaagacaggaatcctaaaagggagagttattactggccacaagccctgtattctcaacagggatgcaaattggttcttcagtaaggataaaaaaaaatcacaagcagttgtttgtggccctcctaaggcccacagcacatatagtgtgtctgtgatattccattttcatggcagggagtgatcaggaagaaggcttcctaggggactggcgatttaaaccagttgagaaacactgccatcagcaggcagtttcagactcactcaagttgtctcttgacagtcacttctaaatgggttctaatgtgacaatggcctccaaaactacagccttccctgaagtttaagctgtgaccttagattttagaaggacagtggggctgtacctagaatagtggttctcgaagaatgcggcctgcagatcctgggagtcccaagaccctttcagggaggatctgtgaggtcaactgttggcactgtggcatgaatcaaggtggtggcagcaaacttctagtagttttgatatgtccttgatagaacaaatagcaatggttaactattaaatgttgacctagccagcgcagtggctcatgcctgtaatcccagcactttgggaggctgaggcgggcggatcacctgaggtcgggagttcgaggccagcctgaccaacatggagaaaccccgtctcttctaaaaatacaaaattagctgggcatggtggtgcatgcctgtaattccagctactcgggaggctgaggcaagagaatcgcttgaatccggtaggtggaggttgcagtgagccgagatcataccattgcactccagcccaggcaacaagagtgaaaccctgtctcaaaaagaaaaaaaaagttgaccttgagaatttataatattctgagaaaactggaagcatgcataaagcccctctgctgtgcactgaagtatgggtgccttgaggaaaagcagttacacagttgagttgcaagctgaattggctgtgttcaaggcatgccctttagaattgaaagaactagcagattacggtatttagacttgaatatttggctgatattttctggaaattaatggaatgagcctctcacctcaagggaaacaactgatagtgttgccagtgataaagctttcaagcaaaaattggaatttccgaaaatctgtactccaccatgagctttattgttggggatattaacaaatgtgatttgtataatgaaatgcatttcatttggaagaattcaatgaaccatttttccaagtgaccagtacgtgatgttacaaaatcatgcatggctcaaagattgattcaaaagtgtaagacaggccagtggattttaatgtattaacaatataagagtgcattaagttttcggagtctacattgcctttaagaaactatgacttgtagtaagccgggcgcggtggctcacgcctgtaatcccaacactttgggaggccaaggtgggtggatcacaaggtcaggagttcaagaccagcctggccaatatggtgaaagtccgtctctactaaaattacaaaaattagccgggcgtggtggcagatcccttgtagtcccagctactcgggaggctgaggcaggagaatagcttgaacccgggaggtggaggttgcagtgagtcgagatcgtgccactggactccagcctgggtgacagagcgagactccatttcaaaaaaaaaaaaaaaaaaaaaaaatcacttgtagtcttggtgtggtatcaaagaatagccacaattagctgaaaaggctattttaaaaacttttccaactgcgtatctgtgtgaagtcaacttacttcaacaaaaaagtttggatgtagaagcagctgtaagaattcaactgtttattataacaagatactaaagagactgtaaaatgccacccttctccttggattgttttggaagttattcttcataaaaaatgttaacgtgggctgggcatggtggctcatgcctgtaatcccagcactctgggaggctgaggtgggcggatcacttgagctcaggaattcaaggtcagcctgggcaacatggctaaactctgtctctattaagaaaaaaaatgttaacattatgatttaaaagtgcattaaccttaatctagataataaaagctttttggggcaacctccagaactgtgaaaaataaatttgttatttaaaaagaaaaaaaaaaaaa

SEQ ID NO: 10 - protein, 339 aa, Homo sapiens
MKDSLVLLGRVPAHPDSRCWFLAWNPAGTLLASCGGDRRIRIWGTEGDSWICKSVLSEGHQRTVRKVAWSPCGNYLASASFDATTCIWKKNQDDFECVTTLEGHENEVKSVAWAPSGNLLATCSRDKSVWVWEVDEEDEYECVSVLNSHTQDVKHVVWHPSQELLASASYDDTVKLYREEEDDWVCCATLEGHESTVWSLAFDPSGQRLASCSDDRTVRIWRQYLPGNEQGVACSGSDPSWKCICTLSGFHSRTIYDIAWCQLTGALATACGDDAIRVFQEDPNSDPQQPTFSLTAHLHQAHSQDVNCVAWNPKEPGLLASCSDDGEVAFWKYQRPEGL

SEQ ID NO: 11 - DNA, 2224 bp, Homo sapiens
  source 1..2224: mol_type = genomic DNA
ggatccgggccgcgcttcctctcgccaggcctgcgagcttcctcccagcggagccctgggcgagccgaggccgctgatgccgcccgcggcgaggtggcccggaccgcagtgccccaagagagctctaatggtaccaagtgacaggttggctttactgtgactcggggacgccagagctcctgagaagatgtcagcaatacaggccgcctggccatccggtacagaatgtattgccaagtacaacttccacggcactgccgagcaggacctgcccttctgcaaaggagacgtgctcaccattgtggccgtcaccaaggaccccaactggtacaaagccaaaaacaaggtgggccgtgagggcatcatcccagccaactacgtccagaagcgggagggcgtgaaggcgggtaccaaactcagcctcatgccttggttccacggcaagatcacacgggagcaggctgagcggcttctgtacccgccggagacaggcctgttcctggtgcgggagagcaccaactaccccggagactacacgctgtgcgtgagctgcgacggcaaggtggagcactaccgcatcatgtaccatgccagcaagctcagcatcgacgaggaggtgtactttgagaacctcatgcagctggtggagcactacacctcagacgcagatggactctgtacgcgcctcattaaaccaaaggtcatggagggcacagtggcggcccaggatgagttctaccgcagcggctgggccctgaacatgaaggagctgaagctgctgcagaccatcgggaagggggagttcggagacgtgatgctgggcgattaccgagggaacaaagtcgccgtcaagtgcattaagaacgacgccactgcccaggccttcctggctgaagcctcagtcatgacgcaactgcggcatagcaacctggtgcagctcctgggcgtgatcgtggaggagaagggcgggctctacatcgtcactgagtacatggccaaggggagccttgtggactacctgcggtctaggggtcggtcagtgctgggcggagactgtctcctcaagttctcgctagatgtctgcgaggccatggaatacctggagggcaacaatttcgtgcatcgagacctggctgcccgcaatgtgctggtgtctgaggacaacgtggccaaggtcagcgactttggtctcaccaaggaggcgtccagcacccaggacacgggcaagctgccagtcaagtggacagcccctgaggccctgagagagaagaaattctccactaagtctgacgtgtggagtttcggaatccttctctgggaaatctactcctttgggcgagtgccttatccaagaattcccctgaaggacgtcgtccctcgggtggagaagggctacaagatggatgcccccgacggctgcccgcccgcagtctatgaagtcatgaagaactgctggcacctggacgccgccatgcggccctccttcctacagctccgagagcagcttgagcacatcaaaacccacgagctgcacctgtgacggctggcctccgcctgggtcatgggcctgtggggactgaacctggaagatcatggacctggtgcccctgctcactgggcccgagcctgaactgagccccagcgggctggcgggcctttttcctgcgtcccagcctgcacccctccggccccgtctctcttggacccacctgtggggcctggggagcccactgaggggccagggaggaaggaggccacggagcgggaggcagcgccccaccacgtcgggcttccctggcctcccgccactcgccttcttagagttttattcctttccttttttgagattttttttccgtgtgtttattttttattatttttcaagataaggagaaagaaagtacccagcaaatgggcattttacaagaagtacgaatcttatttttcctgtcctgcccgtgagggtgggggggaccgggcccctctctagggacccctcgccccagcctcattccccattctgtgtcccatgtcccgtgtctcctcggtcgccccgtgtttgcgcttgaccatgttgcactgtttgcatgcgcccgaggcagacgtctgtcaggggcttggatttcgtgtgccgctgccacccgcccacccgccttgtgagatggaattgtaataaaccacgccatgaggacaccgccgcccgcctcggcgcttcctccaccga

SEQ ID NO: 12 - protein, 450 aa, Homo sapiens
MSAIQAAWPSGTECIAKYNFHGTAEQDLPFCKGDVLTIVAVTKDPNWYKAKNKVGREGIIPANYVQKREGVKAGTKLSLMPWFHGKITREQAERLLYPPETGLFLVRESTNYPGDYTLCVSCDGKVEHYRIMYHASKLSIDEEVYFENLMQLVEHYTSDADGLCTRLIKPKVMEGTVAAQDEFYRSGWALNMKELKLLQTIGKGEFGDVMLGDYRGNKVAVKCIKNDATAQAFLAEASVMTQLRHSNLVQLLGVIVEEKGGLYIVTEYMAKGSLVDYLRSRGRSVLGGDCLLKFSLDVCEAMEYLEGNNFVHRDLAARNVLVSEDNVAKVSDFGLTKEASSTQDTGKLPVKWTAPEALREKKFSTKSDVWSFGILLWEIYSFGRVPYPRIPLKDVVPRVEKGYKMDAPDGCPPAVYEVMKNCWHLDAAMRPSFLQLREQLEHIKTHELHL

SEQ ID NO: 13 - DNA, 3052 bp, Homo sapiens
  source 1..3052: mol_type = genomic DNA
actcggcggacgcaagggcggcggggagcacacggagcactgcaggcgccgggttgggacagcgtcttcgctgctgctggatagtcgtgttttcggggatcgaggatactcaccagaaaccgaaaatgccgaaaccaatcaatgtccgagttaccaccatggatgcagagctggagtttgcaatccagccaaatacaactggaaaacagctttttgatcaggtggtaaagactatcggcctccgggaagtgtggtactttggcctccactatgtggataataaaggatttcctacctggctgaagctggataagaaggtgtctgcccaggaggtcaggaaggagaatcccctccagttcaagttccgggccaagttctaccctgaagatgtggctgaggagctcatccaggacatcacccagaaacttttcttcctccaagtgaaggaaggaatccttagcgatgagatctactgcccccctgagactgccgtgctcttggggtcctacgctgtgcaggccaagtttggggactacaacaaagaagtgcacaagtctgggtacctcagctctgagcggctgatccctcaaagagtgatggaccagcacaaacttaccagggaccagtgggaggaccggatccaggtgtggcatgcggaacaccgtgggatgctcaaagataatgctatgttggaatacctgaagattgctcaggacctggaaatgtatggaatcaactatttcgagataaaaaacaagaaaggaacagacctttggcttggagttgatgcccttggactgaatatttatgagaaagatgataagttaaccccaaagattggctttccttggagtgaaatcaggaacatctctttcaatgacaaaaagtttgtcattaaacccatcgacaagaaggcacctgactttgtgttttatgccccacgtctgagaatcaacaagcggatcctgcagctctgcatgggcaaccatgagttgtatatgcgccgcaggaagcctgacaccatcgaggtgcagcagatgaaggcccaggcccgggaggagaagcatcagaagcagctggagcggcaacagctggaaacagagaagaaaaggagagaaaccgtggagagagagaaagagcagatgatgcgcgagaaggaggagttgatgctgcggctgcaggactatgaggagaagacaaagaaggcagagagagagctctcggagcagattcagagggccctgcagctggaggaggagaggaagcgggcacaggaggaggccgagcgcctagaggctgaccgtatggctgcactgcgggctaaggaggagctggagagacaggcggtggatcagataaagagccaggagcagctggctgcggagcttgcagaatacactgccaagattgccctcctggaagaggcgcggaggcgcaaggaggatgaagttgaagagtggcagcacagggccaaagaagcccaggatgacctggtgaagaccaaggaggagctgcacctggtgatgacagcacccccgcccccaccaccccccgtgtacgagccggtgagctaccatgtccaggagagcttgcaggatgagggcgcagagcccacgggctacagcgcggagctgtctagtgagggcatccgggatgaccgcaatgaggagaagcgcatcactgaggcagagaagaacgagcgtgtgcagcggcagctgctgacgctgagcagcgagctgtcccaggcccgagatgagaataagaggacccacaatgacatcatccacaacgagaacatgaggcaaggccgggacaagtacaagacgctgcggcagatccggcagggcaacaccaagcagcgcatcgacgagttcgaggccctgtaacagccaggccaggaccaagggcagaggggtgctcatagcgggcgctgccagccccgccacgcttgtgtctttagtgctccaagtctaggaactccctcagatcccagttcctttagaaagcagttacccaacagaaacattctgggctgggaaccagggaggcgccctggtttgttttccccagttgtaatagtgccaagcaggcctgattctcgcgattattctcgaatcacctcctgtgttgtgctgggagcaggactgattgaattacggaaaatgcctgtaaagtctgagtaagaaacttcatgctggcctgtgtgatacaagagtcagcatcattaaaggaaacgtggcaggacttccatctgtgccatacttgttctgtattcgaaatgagctcaaattgattttttaatttctatgaaggatccatctttgtatatttacatgcttagaggggtgaaaattattttggaaattgagtctgaagcactctcgcacacacagtgattccctcctcccgtcactccacgcagctggcagagagcacagtgatcaccagcgtgagtggtggaggaggacacttggatttttttttttgttttttttttttttgcttaacagttttagaatacattgtacttatacaccttattaatgatcagctatatactatttatatacaagtgataatacagatttgtaacattagttttaaaaagggaaagttttgttctgtatattttgttaccttttacagaataaaagaattacatatgaaaaaccctctaaaccatggcacttgatgtgatgtggcaggagggcagtggtggagctggacctgcctgctgcagtcacgtgtaaacaggattattattagtgttttatgcatgtaatggactatgcacacttttaattttgtcagattcacacatgccactatgagctttcagactccagctgtgaagagactctgtttgcttgtgtttgtttgtttgcagtctctctctgccatggccttggcaggctgctggaaggcagcttgtggaggccgttggttccgcccactcattccttctcgtgcactgctttctccttcacagctaagatgccatgtgcaggtggattccatgccgcagacatgaaataaaagctttgcaaaggca

SEQ ID NO: 14 - protein, 586 aa, Homo sapiens
MPKPINVRVTTMDAELEFAIQPNTTGKQLFDQVVKTIGLREVWYFGLHYVDNKGFPTWLKLDKKVSAQEVRKENPLQFKFRAKFYPEDVAEELIQDITQKLFFLQVKEGILSDEIYCPPETAVLLGSYAVQAKFGDYNKEVHKSGYLSSERLIPQRVMDQHKLTRDQWEDRIQVWHAEHRGMLKDNAMLEYLKIAQDLEMYGINYFEIKNKKGTDLWLGVDALGLNIYEKDDKLTPKIGFPWSEIRNISFNDKKFVIKPIDKKAPDFVFYAPRLRINKRILQLCMGNHELYMRRRKPDTIEVQQMKAQAREEKHQKQLERQQLETEKKRRETVEREKEQMMREKEELMLRLQDYEEKTKKAERELSEQIQRALQLEEERKRAQEEAERLEADRMAALRAKEELERQAVDQIKSQEQLAAELAEYTAKIALLEEARRRKEDEVEEWQHRAKEAQDDLVKTKEELHLVMTAPPPPPPPVYEPVSYHVQESLQDEGAEPTGYSAELSSEGIRDDRNEEKRITEAEKNERVQRQLLTLSSELSQARDENKRTHNDIIHNENMRQGRDKYKTLRQIRQGNTKQRIDEFEAL

SEQ ID NO: 15 - DNA, 6046 bp, Homo sapiens
  source 1..6046: mol_type = genomic DNA
acagtgccaataccatgaagaggagctcagacagctcttaccacatgatacaagagccggctggtggaagagtggggaccagaaagagaatttgctgaagaggagaaggaaaaaaaaaacaccaaaaaaaaaaataaaaaaatccacacacacaaaaaaacctgcgcgtgaggggggaggaaaagcagggccttttaaaaaggcaatcacaacaacttttgctgccaggatgcccttgctttggctgagaggatttctgttggcaagttgctggattatagtgaggagttcccccaccccaggatccgaggggcacagcgcggcccccgactgtccgtcctgtgcgctggccgccctcccaaaggatgtacccaactctcagccagagatggtggaggccgtcaagaagcacattttaaacatgctgcacttgaagaagagacccgatgtcacccagccggtacccaaggcggcgcttctgaacgcgatcagaaagcttcatgtgggcaaagtcggggagaacgggtatgtggagatagaggatgacattggaaggagggcagaaatgaatgaacttatggagcagacctcggagatcatcacgtttgccgagtcaggaacagccaggaagacgctgcacttcgagatttccaaggaaggcagtgacctgtcagtggtggagcgtgcagaagtctggctcttcctaaaagtccccaaggccaacaggaccaggaccaaagtcaccatccgcctcttccagcagcagaagcacccgcagggcagcttggacacaggggaagaggccgaggaagtgggcttaaagggggagaggagtgaactgttgctctctgaaaaagtagtagacgctcggaagagcacctggcatgtcttccctgtctccagcagcatccagcggttgctggaccagggcaagagctccctggacgttcggattgcctgtgagcagtgccaggagagtggcgccagcttggttctcctgggcaagaagaagaagaaagaagaggagggggaagggaaaaagaagggcggaggtgaaggtggggcaggagcagatgaggaaaaggagcagtcgcacagacctttcctcatgctgcaggcccggcagtctgaagaccaccctcatcgccggcgtcggcggggcttggagtgtgatggcaaggtcaacatctgctgtaagaaacagttctttgtcagtttcaaggacatcggctggaatgactggatcattgctccctctggctatcatgccaactactgcgagggtgagtgcccgagccatatagcaggcacgtccgggtcctcactgtccttccactcaacagtcatcaaccactaccgcatgcggggccatagcccctttgccaacctcaaatcgtgctgtgtgcccaccaagctgagacccatgtccatgttgtactatgatgatggtcaaaacatcatcaaaaaggacattcagaacatgatcgtggaggagtgtgggtgctcatagagttgcccagcccagggggaaagggagcaagagttgtccagagaagacagtggcaaaatgaagaaatttttaaggtttctgagttaaccagaaaaatagaaattaaaaacaaaacaaaaaaaaaaacaaaaaaaaacaaaagtaaattaaaaacaaaacctgatgaaacagatgaaggaagatgtggaaaaaatccttagccagggctcagagatgaagcagtgaaagagacaggaattgggagggaaagggagaatggtgtaccctttatttcttctgaaatcacactgatgacatcagttgtttaaacggggtattgtcctttccccccttgaggttcccttgtgagccttgaatcaaccaatctagtctgcagtagtgtggactagaacaacccaaatagcatctagaaagccatgagtttgaaagggcccatcacaggcactttcctacccaattacccaggtcataaggtatgtctgtgtgacacttatctctgtgtatatcagcatacacacacacacacacacacacacacacacacacaggcatttccacacattacatatatacacatactggtaaaagaacaatcgtgtgcaggtggtcacacttcctttttctgtaccacttttgcaacaaaacaaaacaaacaacattaaaaaattgagaacaagtatggaaagaatgaaagatcaaggaaaaaagaataccaagttacatttcgttaaggtgcttatgatcttagaactatgcaacctaataggtttgaaactgtttacctgagagagaacaaaaagagagacttttttgtattggaagtaatctgattaatttttattttcttcaaggagagatacttgaaaggaatatgtttgtccatctgttggatccaaacatttctatattttgtaaatgttgttgttgttttttttttaatcgtttactatttgcactacaatggtgtttgacctgtctaatccttatttaacaagtattttctttggttgggggtgggggtggggtttaagagctgcacttaatgtgagctataaaagaactgctacagcacacaaaatagctatttttattattataattataattattattattattttgtaccttaaaaaatagacacatacaccaaagacatttgtgtgagcctttaaacagtctgtctgtggttggtatcattcaccatcaatgagtcaggggttgggattcaaggttgagtagtgtggattgtgttcaggcttaaaagacctgagaagtttggtttttgactccttttacatccatgaaacaggacatttcatactggatgtacagtagttgtacactgttggatatcaagttcaatcaaattcatggaactacatgcttgtatgtgtatatatacattgcttgtgcatatgcatatctgtatgtatatatacatgtattgtaccatgtccatacacattttaagcacttcaggctgtcattttttaatgttcttaaagcaatgaatgtttgtgtgcaaaacacagtatttttaagaaggataggctatagtttttgcttttactctgaactaggtgggcgcatttcaaaaattcggatgggaaaaagcctggaaattccagtgaatattcagcaaggccctctttcattgtacagggatcaaatttcctcctcttttttgtgccccctcccacttctacaagttatcccctgtggggaaaacaggatgataatcaaaactctgggctgatgtttttccaacttagtgtctattggaatcaatcttaaatcagaagctttttcagaaaaataatatttaggccagaattagagttgagtgtattttttaaaaatgattaaggcttggttgtgagaaatattacctgtaccagctgggaaaaataatgtcatcactaactaaaagataattaatttgagagaaagtgttaagagagggagagtaaggaagagaacagttaagaggaggcagaggtgagggcagtagtaaaaatctctaaaattttaatttacagccaaaattcttcatgtgtaaatttgtattgattcagatgcagaaatgaaaaaaaaacacctttgttttataaatatcaaagtacatgcttaaagccaagtttttatctagtttattctagtacttagcttgcctggaatagctaataaattattcatgtatgtgcttttgaaaatccagagccctatttttacacacttgtgtgaagttggcaaacattttgaaaaatggaaaaaagtttctaataattgggaacaattacattaattaatattttgtaaaatattgaagcttttagccctatgtcaatttgtagattaaaataaattaattataggaaaggaagataacagtgagaaaccaaacattacaaaaggtggtttagctctccttgaaaaatatactaagttggtatactataacacttggctatatgtaggcaatgtcactactgggcaaatacacttactgtgttctagaggcagccctttcttatgcagaaaatacaatacgcactgcatgagaagcttgagagtggattctaatccaggtctgtcgaccttggatatcatgcatgtgggaaggtgggtgtggtgagaaaagttttaaggcaagagtagatggccatgttcaactttacaaaatttcttggaaaactggcagtattttgaactgcatcttctttggtaccggaacctgcagaaacagtgtgagaaattaagtcctggttcactgcgcagtagcaaagatggtcaaggccatggaaaaagcagaaatttaccaagaaagctgatacccatgtatagttcccactcatctcaaatacatctgctatctttttaagctaagtcctagacatatcggggataacatgggggttgattagtgaccacagttatcagaagcagagaaatgtaattccatattttatttgaaacttattccatattttaattggatattgagtgattgggttatcaaacacccacaaactttaattttgttaaatttatatggctttgaaatagaagtataagttgctaccattttttgataacattgaaagatagtattttaccatctttaatcatcttggaaaatacaagtcctgtgaacaaccactctttcacctagcagcatgaggccaaaagtaaaggctttaaattataacatatgggattcttagtagtatgtttttttcttgaaactcagtggctctatctaaccttactatctcctcactctttctctaagactaaactctaggctcttaaaaatctgcccacaccaatcttagaagctctgaaaagaatttgtctttaaatatcttttaatagtaacatgtattttatggaccaaattgacattttcgactattttttccaaaaaagtcaggtgaatttcagcacactgagttgggaatttcttatcccagaagaccaaccaatttcatatttatttaagattgattccatactccgttttcaaggagaatccctgcagtctccttaaaggtagaacaaatactttctatttttttttcaccattgtgggattggactttaagaggtgactctaaaaaaacagagaacaaatatgtctcagttgtattaagcacggacccatattatcatattcacttaaaaaaatgatttcctgtgcaccttttggcaacttctcttttcaatgtagggaaaaacttagtcaccctgaaaacccacaaaataaataaaacttgtagatgtgggcagaaggtttgggggtggacattgtatgtgtttaaattaaaccctgtatcactgagaagctgttgtatgggtcagagaaaatgaatgcttagaagctgttcacatcttcaagagcagaagcaaaccacatgtctcagctatattattatttattttttatgcataaagtgaatcatttcttctgtattaatttccaaagggttttaccctctatttaaatgctttgaaaaacagtgcattgacaatgggttgatatttttctttaaaagaaaaatataattatgaaagccaagataatctgaagcctgttttattttaaaactttttatgttctgtggttgatgttgtttgtttgtttgtttctattttgttggttttttactttgttttttgttttgttttgttttgttttgcatactacatgcagttctttaaccaatgtctgtttggctaatgtaattaaagttgttaatttatatgagtgcatttcaactatgtcaatggtttcttaatatttattgtgtagaagtactggtaatttttttatttacaatatgtttaaagagataacagtttgatatgttttcatgtgtttatagcagaagttatttatttctatggcattccagcggatattttggtgtttgcgaggcatgcagtcaatattttgtacagttagtggacagtattcagcaacgcctgatagcttctttggccttatgttaaataaaaagacctgtttgggatgta

SEQ ID NO: 16 - protein, 426 aa, Homo sapiens
MPLLWLRGFLLASCWIIVRSSPTPGSEGHSAAPDCPSCALAALPKDVPNSQPEMVEAVKKHILNMLHLKKRPDVTQPVPKAALLNAIRKLHVGKVGENGYVEIEDDIGRRAEMNELMEQTSEIITFAESGTARKTLHFEISKEGSDLSVVERAEVWLFLKVPKANRTRTKVTIRLFQQQKHPQGSLDTGEEAEEVGLKGERSELLLSEKVVDARKSTWHVFPVSSSIQRLLDQGKSSLDVRIACEQCQESGASLVLLGKKKKKEEEGEGKKKGGGEGGAGADEEKEQSHRPFLMLQARQSEDHPHRRRRRGLECDGKVNICCKKQFFVSFKDIGWNDWIIAPSGYHANYCEGECPSHIAGTSGSSLSFHSTVINHYRMRGHSPFANLKSCCVPTKLRPMSMLYYDDGQNIIKKDIQNMIVEECGCS